European Patent Application EP 4 382 911 A1, published June 12, 2024. Title: METHODS FOR SCREENING AND DIAGNOSING CANCER. Applicant: Oncomatryx Biopharma, S.L. Application EP. The sequence listing filed with the application follows.

SEQUENCE LISTING (18 sequences)

SEQ ID NO: 1 - DNA, 22 bp, synthetic construct
  source 1..22: mol_type = other DNA
cagccactactacacgaccatc

SEQ ID NO: 2 - DNA, 22 bp, synthetic construct
  source 1..22: mol_type = other DNA
caaacttggttcggaagtcatc

SEQ ID NO: 3 - DNA, 20 bp, synthetic construct
  source 1..20: mol_type = other DNA
cagccagacgggcattgtcg

SEQ ID NO: 4 - DNA, 18 bp, synthetic construct
  source 1..18: mol_type = other DNA
cctggaccaatgggctta

SEQ ID NO: 5 - DNA, 18 bp, synthetic construct
  source 1..18: mol_type = other DNA
gaaaccttgagggcctgg

SEQ ID NO: 6 - DNA, 21 bp, synthetic construct
  source 1..21: mol_type = other DNA
tagaggcccacctggtgcagc

SEQ ID NO: 7 - DNA, 20 bp, synthetic construct
  source 1..20: mol_type = other DNA
ccacactgtgcccatctacg

SEQ ID NO: 8 - DNA, 26 bp, synthetic construct
  source 1..26: mol_type = other DNA
aggatcttcatgaggtagtcagtcag

SEQ ID NO: 9 - DNA, 21 bp, synthetic construct
  source 1..21: mol_type = other DNA
caggtccagacgcaggatggc

SEQ ID NO: 10 - DNA, 17 bp, synthetic construct
  source 1..17: mol_type = other DNA
agcctcgcctttgccga

SEQ ID NO: 11 - DNA, 15 bp, synthetic construct
  source 1..15: mol_type = other DNA
ctggtgcctggggcg

SEQ ID NO: 12 - DNA, 19 bp, synthetic construct
  source 1..19: mol_type = other DNA
aatgggataccgcagcaac

SEQ ID NO: 13 - DNA, 24 bp, synthetic construct
  source 1..24: mol_type = other DNA
gagagaccaggagaagttccagat

SEQ ID NO: 14 - DNA, 20 bp, synthetic construct
  source 1..20: mol_type = other DNA
aatggagctgatggaccaca

SEQ ID NO: 15 - DNA, 18 bp, synthetic construct
  source 1..18: mol_type = other DNA
tcctttgggaccgcctac

SEQ ID NO: 16 - DNA, 19 bp, synthetic construct
  source 1..19: mol_type = other DNA
tcaaactggctgccagcat

SEQ ID NO: 17 - DNA, 21 bp, synthetic construct
  source 1..21: mol_type = other DNA
caagaaacacgtctggctagg

SEQ ID NO: 18 - DNA, 25 bp, synthetic construct
  source 1..25: mol_type = other DNA
ctccaacaccaccaactgaaccaac